European Patent Application EP 4 183 798 A1, published May 24, 2023. Title: COMPOSITIONS AND METHODS FOR TREATING CANCER WITH ANTI-MESOTHELIN IMMUNOTHERAPY. Applicant: Lentigen Technology, Inc. Application EP 21160649.6, filed January 9, 2018. The sequence listing filed with the application follows.

SEQUENCE LISTING (30 sequences)

SEQ ID NO: 1 - DNA, 738 bp, synthetic construct
  misc_feature 1..738: note = mesothelin antigen ScFv binding domain MH1P
  source 1..738: mol_type = other DNA
caggtacagctgcagcagtcaggtccaggactggtgaagccctcgcggaccctctcactcacctgtgccatctccggggacagtgtctctagcaacagtgctgcttggaactggatcaggcagtccccatcgagaggccttgagtggctgggaaggacatactacaggtccaagtggtataatgattatgcagtatctgtgaaaagtcgaataaccatcaacccagacacatccaagaaccagttctccctgcagctgaactctgtgactcccgaggacacggctgtgtattactgtgcaagagggaagggtggtaagaagggtggtgcttttgatatctggggccaagggacaatggtcaccgtctcttcaggaggtggcgggtctggtggaggcggtagcggcggtggcggatcctcttctgagctgactcaggaccctgctgtgtctgtggccttgggacagacagtcaggatcacatgccaaggagacagcctcagaagctattatgcaagctggtaccagcagaagccaggacaggctcctgtacttgtcatctatggtaaaaacaaccggccctcagggatcccagaccgattctctggctcctcctcaggcaacacagcttccttgaccatcactggggctcaggcggaagatgaggctgaatattactgtagctccagcactcgtaatcatgtgttcttcggcagagggaccaaggtcaccgtcctaggt

SEQ ID NO: 2 - protein, 245 aa, synthetic construct
  REGION 1..245: note = mesothelin antigen ScFv binding domain MH1P
QVQLQSGPGLVKPSRTLSLTCAISGDSVSSNSAAWNWIRQSPSRGLEWLGRTYYRSKWYNDYAVSVKSRITINPDTSKNQFSLQLNSVTPEDTAVYYCARGKGGKKGGAFDIWGQGTMVTVSSGGGGSGGGGSGGGGSSSELTQDPAVSVALGQTVRITCQGDSLRSYYASWYQQKPGQAPVLVIYGKNNRPSGIPDRFSGSSSGNTASLTITGAQAEDEAEYYCSSSTRNHVFFGRGTKVTVLG

SEQ ID NO: 3 - DNA, 735 bp, synthetic construct
  misc_feature 1..735: note = mesothelin antigen ScFv binding domain MH2P
  source 1..735: mol_type = other DNA
gaggtgcagctggtgcagtctgggggaggcttggtacagcctggcaggtcccagagactctcctgtgcagcctctggattcacctttgatgattatgccatgcactgggtccggcaagctccagggaagggcctggagtgggtctcaggtattagttggaatagtggtagcataggctatgcggactctgtgaagggccgattcaccatctccagagacaacgccaagaactccctgtatctgcaaatgaacagtctgagagctgaggacacggccttgtattactgtgcaaaagatatttcgtcgtcagctggtaacgcttttgatatctggggccaagggacaatggtcaccgtctcttcaggaggtggcgggtctggtggaggcggtagcggcggtggcggatcctcttctgagctgactcaggaccctgctgtgtctgtggccttgggacagacagtcaggatcacatgccaaggagacagactcagaagctattatgcaagctggtaccagcagaagccaggacaggcccctgtacttgtcatctatggtaaaaacaaccggccctcagggatcccagaccgcttctctggctccgactcaggagacacagcttccttgaccatcactggggctcaggcggaagatgaggctgactattactgtcactcccgtgacagtggtggtaaccatgtggtattcggcggaggcacccagctgaccgtcctcggt

SEQ ID NO: 4 - protein, 245 aa, synthetic construct
  REGION 1..245: note = mesothelin antigen ScFv binding domain MH2P
EVQLVQSGGGLVQPGRSQRLSCAASGFTFDDYAMHWVRQAPGKGLEWVSGISWNSGSIGYADSVKGRFTISRDNAKNSLYLQMNSLRAEDTALYYCAKDISSSAGNAFDIWGQGTMVTVSSGGGGSGGGGSGGGGSSSELTQDPAVSVALGQTVRITCQGDRLRSYYASWYQQKPGQAPVLVIYGKNNRPSGIPDRFSGSDSGDTASLTITGAQAEDEADYYCHSRDSGGNHVVFGGGTQLTVLG

SEQ ID NO: 5 - DNA, 732 bp, synthetic construct
  misc_feature 1..732: note = mesothelin antigen ScFv binding domain M1-4S
  source 1..732: mol_type = other DNA
gaggtccagctggtacagtctgggggaggcttggtacagcctggggggtccctgagactctcctgtgcagcctctggattcacctttgatgattatgccatgcactgggtccggcaagctccagggaagggcctggagtgggtctcaggtattagttggaatagtggtagcataggctatgcggactctgtgaagggccgattcaccatctccagagacaacgccaagaactccctgtatctgcaaatgaacagtctgagagctgaggacacggccttgtattactgtgcaaaagatttatcgtcagtggctggaccctttaactactggggccagggcaccctggtcaccgtctcctcaggaggtggcgggtctggtggaggcggtagcggcggtggcggatcctcttctgagctgactcaggaccctgctgtgtctgtggccttgggacagacagtcaggatcacatgccaaggagacagcctcagaagctattatgcaagctggtaccagcagaagccaggacaggcccctgtacttgtcatctatggtaaaaacaaccggccctcagggatcccagaccgattctctggctccagctcaggaaacacagcttccttgaccatcactggggctcaggcggaggatgaggctgactattactgtaactcccgggacagcagtggtaaccatctggtattcggcggaggcacccagctgaccgtcctcggt

SEQ ID NO: 6 - protein, 244 aa, synthetic construct
  REGION 1..244: note = mesothelin antigen ScFv binding domain M1-4S
EVQLVQSGGGLVQPGGSLRLSCAASGFTFDDYAMHWVRQAPGKGLEWVSGISWNSGSIGYADSVKGRFTISRDNAKNSLYLQMNSLRAEDTALYYCAKDLSSVAGPFNYWGQGTLVTVSSGGGGSGGGGSGGGGSSSELTQDPAVSVALGQTVRITCQGDSLRSYYASWYQQKPGQAPVLVIYGKNNRPSGIPDRFSGSSSGNTASLTITGAQAEDEADYYCNSRDSSGNHLVFGGGTQLTVLG

SEQ ID NO: 7 - DNA, 732 bp, synthetic construct
  misc_feature 1..732: note = mesothelin antigen ScFv binding domain MH6P
  source 1..732: mol_type = other DNA
caggtccagctggtgcagtctggggctgaggtgaagaagcctggggcctcagtgaaggtctcctgcaaggcttctggatacaccttcaccggctactatatgcactgggtgcgacaggcccctggacaagggcttgagtggatgggacggatcaaccctaacagtggtggcacaaactatgcacagaagtttcagggcagggtcaccatgaccaggaacacgtccatcagcacagcctacatggagctgagcaggctgagatctgacgacacggccgtgtattactgtgcgagatccggctactactacggtttggacgtctggggccaagggaccacggtcaccgtctcctcaggaggtggcgggtctggtggaggcggtagcggcggtggcggatcccagtctgtgttgacgcagccgccctcagcgtctgggacccccgggcagcgggtcaccatctcttgttctggaagtcgctccaacatcggaagaaacactgtcaactggtatcaacaactcccaggactggcccccaaactcatcatccagaggagtgatcagcggccctcaggggtccctgaccgattctctggctccaagtctgtcacctcagcctccctggccatcagtgggctccggtccgaggatgaggctgattattactgcggaacatgggataacagcctgagtgcttatgtcttcggaactgggaccaagctgaccgtcctaggt

SEQ ID NO: 8 - protein, 244 aa, synthetic construct
  REGION 1..244: note = mesothelin antigen ScFv binding domain MH6P
QVQLVQSGAEVKKPGASVKVSCKASGYTFTGYYMHWVRQAPGQGLEWMGRINPNSGGTNYAQKFQGRVTMTRNTSISTAYMELSRLRSDDTAVYYCARSGYYYGLDVWGQGTTVTVSSGGGGSGSGGSGGGGSQSVLTQPPSASGTPGQRVTISCSGSRSNIGRNTVNWYQQLPGLAPKLIIQRSDQRPSGVPDRFSGSKSVTSASLAISGLRSEDEADYYCGTWDNSLSAYVFGTGTKLTVLG

SEQ ID NO: 9 - DNA, 66 bp, synthetic construct
  misc_feature 1..66: note = leader/signal peptide sequence
  source 1..66: mol_type = other DNA
atgctgctgctggtgaccagcctgctgctgtgcgaactgccgcatccggcgtttctgctgattccg

SEQ ID NO: 10 - protein, 22 aa, synthetic construct
  REGION 1..22: note = leader/signal peptide sequence
MLLLVTSLLLCELPHPAFLLIP

SEQ ID NO: 11 - DNA, 1482 bp, synthetic construct
  misc_feature 1..1482: note = pLTG1901 EF1a MH1P--CD8TM-4-1BB-CD3 zeta
  source 1..1482: mol_type = other DNA
atgctgctgctggtgaccagcctgctgctgtgcgaactgccgcatccggcgtttctgctgattccgcaggtacagctgcagcagtcaggtccaggactggtgaagccctcgcggaccctctcactcacctgtgccatctccggggacagtgtctctagcaacagtgctgcttggaactggatcaggcagtccccatcgagaggccttgagtggctgggaaggacatactacaggtccaagtggtataatgattatgcagtatctgtgaaaagtcgaataaccatcaacccagacacatccaagaaccagttctccctgcagctgaactctgtgactcccgaggacacggctgtgtattactgtgcaagagggaagggtggtaagaagggtggtgcttttgatatctggggccaagggacaatggtcaccgtctcttcaggaggtggcgggtctggtggaggcggtagcggcggtggcggatcctcttctgagctgactcaggaccctgctgtgtctgtggccttgggacagacagtcaggatcacatgccaaggagacagcctcagaagctattatgcaagctggtaccagcagaagccaggacaggctcctgtacttgtcatctatggtaaaaacaaccggccctcagggatcccagaccgattctctggctcctcctcaggcaacacagcttccttgaccatcactggggctcaggcggaagatgaggctgaatattactgtagctccagcactcgtaatcatgtgttcttcggcagagggaccaaggtcaccgtcctcggtgcggccgcaactaccacccctgcccctcggccgccgactccggccccaaccatcgcaagccaacccctctccttgcgccccgaagcttgccgcccggccgcgggtggagccgtgcatacccgggggctggactttgcctgcgatatctacatttgggccccgctggccggcacttgcggcgtgctcctgctgtcgctggtcatcaccctttactgcaagaggggccggaagaagctgctttacatcttcaagcagccgttcatgcggcccgtgcagacgactcaggaagaggacggatgctcgtgcagattccctgaggaggaagaggggggatgcgaactgcgcgtcaagttctcacggtccgccgacgcccccgcatatcaacagggccagaatcagctctacaacgagctgaacctgggaaggagagaggagtacgacgtgctggacaagcgacgcggacgcgacccggagatgggggggaaaccacggcggaaaaaccctcaggaaggactgtacaacgaactccagaaagacaagatggcggaagcctactcagaaatcgggatgaagggagagcggaggaggggaaagggtcacgacgggctgtaccagggactgagcaccgccactaaggatacctacgatgccttgcatatgcaagcactcccaccccgg

SEQ ID NO: 12 - protein, 494 aa, synthetic construct
  REGION 1..494: note = pLTG1901 EF1a MH1P--CD8TM-4-1BB-CD3 zeta
MLLLVTSLLLCELPHPAFLLIPQVQLQQSGPGLVKPSRTLSLTCAISGDSVSSNSAAWNWIRQSPSRGLEWLGRTYYRSKWYNDYAVSVKSRITINPDTSKNQFSLQLNSVTPEDTAVYYCARGKGGKKGGAFDIWGQGTMVTVSSGGGGSGGGGSGGGGSSSELTQDPAVSVALGQTVRITCQGDSLRSYYASWYQQKPGQAPVLVIYGKNNRPSGIPDRFSGSSSGNTASLTITGAQAEDEAEYYCSSSTRNHVFFGRGTKVTVLGAAATTTPAPRPPTPAPTIASQPLSLRPEACRPAAGGAVHTRGLDFACDIYIWAPLAGTCGVLLLSLVITLYCKRGRKKLLYIFKQPFMRPVQTTQEEDGCSCRFPEEEEGGCELRVKFSRSADAPAYQQGQNQLYNELNLGRREEYDVLDKRRGRDPEMGGKPRRKNPQEGLYNELQKDKMAEAYSEIGMKGERRRGKGHDGLYQGLSTATKDTYDALHMQALPPR

SEQ ID NO: 13 - DNA, 1479 bp, synthetic construct
  misc_feature 1..1479: note = pLTG1902 Ef1a MH2P CD8TM-4-1BB-CD3 zeta
  source 1..1479: mol_type = other DNA
atgctgctgctggtgaccagcctgctgctgtgcgaactgccgcatccggcgtttctgctgattccggaggtgcagctggtgcagtctgggggaggcttggtacagcctggcaggtcccagagactctcctgtgcagcctctggattcacctttgatgattatgccatgcactgggtccggcaagctccagggaagggcctggagtgggtctcaggtattagttggaatagtggtagcataggctatgcggactctgtgaagggccgattcaccatctccagagacaacgccaagaactccctgtatctgcaaatgaacagtctgagagctgaggacacggccttgtattactgtgcaaaagatatttcgtcgtcagctggtaacgcttttgatatctggggccaagggacaatggtcaccgtctcttcaggaggtggcgggtctggtggaggcggtagcggcggtggcggatcctcttctgagctgactcaggaccctgctgtgtctgtggccttgggacagacagtcaggatcacatgccaaggagacagactcagaagctattatgcaagctggtaccagcagaagccaggacaggcccctgtacttgtcatctatggtaaaaacaaccggccctcagggatcccagaccgcttctctggctccgactcaggagacacagcttccttgaccatcactggggctcaggcggaagatgaggctgactattactgtcactcccgtgacagtggtggtaaccatgtggtattcggcggaggcacccagctgaccgtcctcggtgcggccgcaactaccacccctgcccctcggccgccgactccggccccaaccatcgcaagccaacccctctccttgcgccccgaagcttgccgcccggccgcgggtggagccgtgcatacccgggggctggactttgcctgcgatatctacatttgggccccgctggccggcacttgcggcgtgctcctgctgtcgctggtcatcaccctttactgcaagaggggccggaagaagctgctttacatcttcaagcagccgttcatgcggcccgtgcagacgactcaggaagaggacggatgctcgtgcagattccctgaggaggaagaggggggatgcgaactgcgcgtcaagttctcacggtccgccgacgcccccgcatatcaacagggccagaatcagctctacaacgagctgaacctgggaaggagagaggagtacgacgtgctggacaagcgacgcggacgcgacccggagatgggggggaaaccacggcggaaaaaccctcaggaaggactgtacaacgaactccagaaagacaagatggcggaagcctactcagaaatcgggatgaagggagagcggaggaggggaaagggtcacgacgggctgtaccagggactgagcaccgccactaaggatacctacgatgccttgcatatgcaagcactcccaccccgg

SEQ ID NO: 14 - protein, 493 aa, synthetic construct
  REGION 1..493: note = pLTG1902 Ef1a MH2P CD8TM-4-1BB-CD3 zeta
MLLLVTSLLLCELPHPAFLLIPEVQLVQSGGGLVQPGRSQRLSCAASGFTFDDYAMHWVRQAPGKGLEWVSGISWNSGSIGYADSVKGRFTISRDNAKNSLYLQMNSLRAEDTALYYCAKDISSSAGNAFDIWGQGTMVTVSSGGGGSGGGGSGGGGSSSELTQDPAVSVALGQTVRITCQGDRLRSYYASWYQQKPGQAPVLVIYGKNNRPSGIPDRFSGSDSGDTASLTITGAQAEDEADYYCHSRDSGGNHVVFGGGTQLTVLGAAATTTPAPRPPTPAPTIASQPLSLRPEACRPAAGGAVHTRGLDFACDIYIWAPLAGTCGVLLLSLVITLYCKRGRKKLLYIFKQPFMRPVQTTQEEDGCSCRFPEEEEGGCELRVKFSRSADAPAYQQGQNQLYNELNLGRREEYDVLDKRRGRDPEMGGKPRRKNPQEGLYNELQKDKMAEAYSEIGMKGERRRGKGHDGLYQGLSTATKDTYDALHMQALPPR

SEQ ID NO: 15 - DNA, 1476 bp, synthetic construct
  misc_feature 1..1476: note = pLTG1903 Ef1a MH6P CD8TM-4-1BB-CD3 zeta
  source 1..1476: mol_type = other DNA
atgctgctgctggtgaccagcctgctgctgtgcgaactgccgcatccggcgtttctgctgattccgcaggtccagctggtgcagtctggggctgaggtgaagaagcctggggcctcagtgaaggtctcctgcaaggcttctggatacaccttcaccggctactatatgcactgggtgcgacaggcccctggacaagggcttgagtggatgggacggatcaaccctaacagtggtggcacaaactatgcacagaagtttcagggcagggtcaccatgaccaggaacacgtccatcagcacagcctacatggagctgagcaggctgagatctgacgacacggccgtgtattactgtgcgagatccggctactactacggtttggacgtctggggccaagggaccacggtcaccgtctcctcaggaggtggcgggtctggtggaggcggtagcggcggtggcggatcccagtctgtgttgacgcagccgccctcagcgtctgggacccccgggcagcgggtcaccatctcttgttctggaagtcgctccaacatcggaagaaacactgtcaactggtatcaacaactcccaggactggcccccaaactcatcatccagaggagtgatcagcggccctcaggggtccctgaccgattctctggctccaagtctgtcacctcagcctccctggccatcagtgggctccggtccgaggatgaggctgattattactgcggaacatgggataacagcctgagtgcttatgtcttcggaactgggaccaagctgaccgtcctcggtgcggccgcaactaccacccctgcccctcggccgccgactccggccccaaccatcgcaagccaacccctctccttgcgccccgaagcttgccgcccggccgcgggtggagccgtgcatacccgggggctggactttgcctgcgatatctacatttgggccccgctggccggcacttgcggcgtgctcctgctgtcgctggtcatcaccctttactgcaagaggggccggaagaagctgctttacatcttcaagcagccgttcatgcggcccgtgcagacgactcaggaagaggacggatgctcgtgcagattccctgaggaggaagaggggggatgcgaactgcgcgtcaagttctcacggtccgccgacgcccccgcatatcaacagggccagaatcagctctacaacgagctgaacctgggaaggagagaggagtacgacgtgctggacaagcgacgcggacgcgacccggagatgggggggaaaccacggcggaaaaaccctcaggaaggactgtacaacgaactccagaaagacaagatggcggaagcctactcagaaatcgggatgaagggagagcggaggaggggaaagggtcacgacgggctgtaccagggactgagcaccgccactaaggatacctacgatgccttgcatatgcaagcactcccaccccgg

SEQ ID NO: 16 - protein, 492 aa, synthetic construct
  REGION 1..492: note = pLTG1903 Ef1a MH6P CD8TM-4-1BB-CD3 zeta
MLLLVTSLLLCELPHPAFLLIPQVQLVQSGAEVKKPGASVKVSCKASGYTFTGYYMHWVRQAPGQGLEWMGRINPNSGGTNYAQKFQGRVTMTRNTSISTAYMELSRLRSDDTAVYYCARSGYYYGLDVWGQGTTVTVSSGGGGSGGGGSGGGGSQSVLTQPPSASGTPGQRVTISCSGSRSNIGRNTVNWYQQLPGLAPKLIIQRSDQRPSGVPDRFSGSKSVTSASLAISGLRSEDEADYYCGTWDNSLSAYVFGTGTKLTVLGAAATTTPAPRPPTPAPTIASQPLSLRPEACRPAAGGAVHTRGLDFACDIYIWAPLAGTCGVLLLSLVITLYCKRGRKKLLYIFKQPFMRPVQTTQEEDGCSCRFPEEEEGGCELRVKFSRSADAPAYQQGQNQLYNELNLGRREEYDVLDKRRGRDPEMGGKPRRKNPQEGLYNELQKDKMAEAYSEIGMKGERRRGKGHDGLYQGLSTATKDTYDALHMQALPPR

SEQ ID NO: 17 - DNA, 1476 bp, synthetic construct
  misc_feature 1..1476: note = pLTG1904 Ef1a M1-4S CD8TM-4-1BB-CD3 zeta
  source 1..1476: mol_type = other DNA
atgctgctgctggtgaccagcctgctgctgtgcgaactgccgcatccggcgtttctgctgattccggaggtccagctggtacagtctgggggaggcttggtacagcctggggggtccctgagactctcctgtgcagcctctggattcacctttgatgattatgccatgcactgggtccggcaagctccagggaagggcctggagtgggtctcaggtattagttggaatagtggtagcataggctatgcggactctgtgaagggccgattcaccatctccagagacaacgccaagaactccctgtatctgcaaatgaacagtctgagagctgaggacacggccttgtattactgtgcaaaagatttatcgtcagtggctggaccctttaactactggggccagggcaccctggtcaccgtctcctcaggaggtggcgggtctggtggaggcggtagcggcggtggcggatcctcttctgagctgactcaggaccctgctgtgtctgtggccttgggacagacagtcaggatcacatgccaaggagacagcctcagaagctattatgcaagctggtaccagcagaagccaggacaggcccctgtacttgtcatctatggtaaaaacaaccggccctcagggatcccagaccgattctctggctccagctcaggaaacacagcttccttgaccatcactggggctcaggcggaggatgaggctgactattactgtaactcccgggacagcagtggtaaccatctggtattcggcggaggcacccagctgaccgtcctcggtgcggccgcaactaccacccctgcccctcggccgccgactccggccccaaccatcgcaagccaacccctctccttgcgccccgaagcttgccgcccggccgcgggtggagccgtgcatacccgggggctggactttgcctgcgatatctacatttgggccccgctggccggcacttgcggcgtgctcctgctgtcgctggtcatcaccctttactgcaagaggggccggaagaagctgctttacatcttcaagcagccgttcatgcggcccgtgcagacgactcaggaagaggacggatgctcgtgcagattccctgaggaggaagaggggggatgcgaactgcgcgtcaagttctcacggtccgccgacgcccccgcatatcaacagggccagaatcagctctacaacgagctgaacctgggaaggagagaggagtacgacgtgctggacaagcgacgcggacgcgacccggagatgggggggaaaccacggcggaaaaaccctcaggaaggactgtacaacgaactccagaaagacaagatggcggaagcctactcagaaatcgggatgaagggagagcggaggaggggaaagggtcacgacgggctgtaccagggactgagcaccgccactaaggatacctacgatgccttgcatatgcaagcactcccaccccgg

SEQ ID NO: 18 - protein, 492 aa, synthetic construct
  REGION 1..492: note = pLTG1904 Ef1a M1-4S CD8TM-4-1BB-CD3 zeta
MLLLVTSLLLCELPHPAFLLIPEVQLVQSGGGLVQPGGSLRLSCAASGFTFDDYAMHWVRQAPGKGLEWVSGISWNSGSIGYADSVKGRFTISRDNAKNSLYLQMNSLRAEDTALYYCAKDLSSVAGPFNYWGQGTLVTVSSGGGGSGGGGSGGGGSSSELTQDPAVSVALGQTVRITCQGDSLRSYYASWYQQKPGQAPVLVIYGKNNRPSGIPDRFSGSSSGNTASLTITGAQAEDEADYYCNSRDSSGNHLVFGGGTQLTVLGAAATTTPAPRPPTPAPTIASQPLSLRPEACRPAAGGAVHTRGLDFACDIYIWAPLAGTCGVLLLSLVITLYCKRGRKKLLYIFKQPFMRPVQTTQEEDGCSCRFPEEEEGGCELRVKFSRSADAPAYQQGQNQLYNELNLGRREEYDVLDKRRGRDPEMGGKPRRKNPQEGLYNELQKDKMAEAYSEIGMKGERRRGKGHDGLYQGLSTATKDTYDALHMQALPPR

SEQ ID NO: 19 - DNA, 72 bp, Homo sapiens
  source 1..72: mol_type = genomic DNA
atctacatctgggcgcccttggccgggacttgtggggtccttctcctgtcactggttatcaccctttactgc

SEQ ID NO: 20 - protein, 22 aa, Homo sapiens
IWAPLAGTCGVLLLSLVITLYC

SEQ ID NO: 21 - DNA, 135 bp, Homo sapiens
  source 1..135: mol_type = genomic DNA
accacgacgccagcgccgcgaccaccaacaccggcgcccaccatcgcgtcgcagcccctgtccctgcgcccagaggcgtgccggccagcggcggggggcgcagtgcacacgagggggctggacttcgcctgtgat

SEQ ID NO: 22 - protein, 47 aa, Homo sapiens
TTTPAPRPPTPAPTIASQPLSLRPEACRPAAGGAVHTRGLDFACDIY

SEQ ID NO: 23 - protein, 42 aa, synthetic construct
  REGION 1..42: note = hinge region of CD8.alpha
KRGRKKLLYIFKQPFMRPVQTTQEEDGCSCRFPEEEEGGCEL

SEQ ID NO: 24 - protein, 106 aa, Homo sapiens
GQPKAAPSVTLFPPSSEELQANKATLVCLISDFYPGAVTVAWKADSSPVKAGVETTTPSKQSNNKYAASSYLSLTPEQWKSHRSYSCQVTHEGSTVEKTVAPTECS

SEQ ID NO: 25 - DNA, 126 bp, Homo sapiens
  source 1..126: mol_type = genomic DNA
aaacggggcagaaagaaactcctgtatatattcaaacaaccatttatgagaccagtacaaactactcaagaggaagatggctgtagctgccgatttccagaagaagaagaaggaggatgtgaactg

SEQ ID NO: 26 - protein, 42 aa, Homo sapiens; identical to SEQ ID NO: 23

SEQ ID NO: 27 - DNA, 336 bp, Homo sapiens
  source 1..336: mol_type = genomic DNA
agagtgaagttcagcaggagcgcagacgcccccgcgtacaagcagggccagaaccagctctataacgagctcaatctaggacgaagagaggagtacgatgttttggacaagagacgtggccgggaccctgagatggggggaaagccgagaaggaagaaccctcaggaaggcctgtacaatgaactgcagaaagataagatggcggaggcctacagtgagattgggatgaaaggcgagcgccggaggggcaaggggcacgatggcctttaccagggtctcagtacagccaccaaggacacctacgacgcccttcacatgcaggccctgccccctcgc

SEQ ID NO: 28 - protein, 112 aa, Homo sapiens
RVKFSRSADAPAYKQGQNQLYNELNLGRREEYDVLDKRRGRDPEMGGKPRRKNPQEGLYNELQKDKMAEAYSEIGMKGERRRGKGHDGLYQGLSTATKDTYDALHMQALPPR

SEQ ID NO: 29 - DNA, 726 bp, synthetic construct
  misc_feature 1..726: note = Scvf cd 19
  source 1..726: mol_type = other DNA
gacatccagatgacacagactacatcctccctgtctgcctctctgggagacagagtcaccatcagttgcagggcaagtcaggacattagtaaatatttaaattggtatcagcagaaaccagatggaactgttaaactcctgatctaccatacatcaagattacactcaggagtcccatcaaggttcagtggcagtgggtctggaacagattattctctcaccattagcaacctggagcaagaagatattgccacttacttttgccaacagggtaatacgcttccgtacacgttcggaggggggaccaagctggagatcacaggtggcggtggctcgggcggtggtgggtcgggtggcggcggatctgaggtgaaactgcaggagtcaggacctggcctggtggcgccctcacagagcctgtccgtcacatgcactgtctcaggggtctcattacccgactatggtgtaagctggattcgccagcctccacgaaagggtctggagtggctgggagtaatatggggtagtgaaaccacatactataattcagctctcaaatccagactgaccatcatcaaggacaactccaagagccaagttttcttaaaaatgaacagtctgcaaactgatgacacagccatttactactgtgccaaacattattactacggtggtagctatgctatggactactggggccaaggaacctcagtcaccgtctcctca

SEQ ID NO: 30 - protein, 242 aa, synthetic construct
  REGION 1..242: note = Scvf cd 19
DIQMTQTTSSLSASLGDRVTISCRASQDISKYLNWYQQKPDGTVKLLIYHTSRLHSGVPSRFSGSGSGTDYSLTISNLEQEDIATYFCQQGNTLPYTFGGGTKLEITGGGGSGGGGSGGGGSEVKLQESGPGLVAPSQSLSVTCTVSGVSLPDYGVSWIRQPPRKGLEWLGVIWGSETTYYNSALKSRLTIIKDNSKSQVFLKMNSLQTDDTAIYYCAKHYYYGGSYAMDYWGQGTSVTVSS